European Patent Specification EP 3 712 262 B1, published May 21, 2025. Title: Transaminase mutant and use thereof. Applicant: ASYMCHEM LIFE SCIENCETIANJIN CO.,LTD. The sequence listing filed with the application follows.

SEQUENCE LISTING (21 sequences)

SEQ ID NO: 1 - protein, 459 aa, Chromobacterium violaceum
MQKQRTTSQWRELDAAHHLHPFTDTASLNQAGARVMTRGEGVYLWDSEGNKIIDGMAGLWCVNVGYGRKDFAEAARRQMEELPFYNTFFKTTHPAVVELSSLLAEVTPAGFDRVFYTNSGSESVDTMIRMVRRYWDVQGKPEKKTLIGRWNGYHGSTIGGASLGGMKYMHEQGDLPIPGMAHIEQPWWYKHGKDMTPDEFGVVAARWLEEKILEIGADKVAAFVGEPIQGAGGVIVPPATYWPEIERICRKYDVLLVADEVICGFGRTGEWFGHQHFGFQPDLFTAAKGLSSGYLPIGAVFVGKRVAEGLIAGGDFNHGFTYSGHPVCAAVAHANVAALRDEGIVQRVKDDIGPYMQKRWRETFSRFEHVDDVRGVGMVQAFTLVKNKAKRELFPDFGEIGTLCRDIFFRNNLIMRACGDHIVSAPPLVMTRAEVDEMLAVAERCLEEFEQTLKARGLA

SEQ ID NO: 2 - DNA, 40 bp, Chromobacterium violaceum
  misc_feature (19)..(20): n is a, c, g, or t
  misc_feature (21)..(21): k is g, or t
ccgttctacaataccttcnnkaaaaccacccacccagctg

SEQ ID NO: 3 - DNA, 40 bp, Chromobacterium violaceum
  misc_feature (20)..(20): m is a or c
  misc_feature (21)..(22): n is a,t, g or c
cagctgggtgggtggttttmnngaaggtattgtagaacgg

SEQ ID NO: 4 - DNA, 42 bp, Chromobacterium violaceum
  misc_feature (20)..(21): n is a, c, g, or t
  misc_feature (22)..(22): k is g or t
gattggccgttggaacggcnnkcacggcagcactattggtgg

SEQ ID NO: 5 - DNA, 42 bp, Chromobacterium violaceum
  misc_feature (21)..(21): m is a, or c
  misc_feature (22)..(23): n is a, c, g, or t
ccaccaatagtgctgccgtgmnngccgttccaacggccaatc

SEQ ID NO: 6 - DNA, 40 bp, Chromobacterium violaceum
  misc_feature (19)..(20): n is a, c, g, or t
  misc_feature (21)..(21): k is g, or t
ggtgagccgatccagggtnnkggtggtgttatcgttccgc

SEQ ID NO: 7 - DNA, 40 bp, Chromobacterium violaceum
  misc_feature (20)..(20): m is a, or c
  misc_feature (21)..(22): n is a, c, g, or t
gcggaacgataacaccaccmnnaccctggatcggctcacc

SEQ ID NO: 8 - DNA, 41 bp, Chromobacterium violaceum
  misc_feature (20)..(21): n is a, c, g, or t
  misc_feature (22)..(22): k is a, or c
cttcaaccacggttttaccnnktctggtcacccagtctgcg

SEQ ID NO: 9 - DNA, 41 bp, Chromobacterium violaceum
  misc_feature (20)..(20): m is a,or c
  misc_feature (21)..(22): n is a, c, g, or t
cgcagactgggtgaccagamnnggtaaaaccgtggttgaag

SEQ ID NO: 10 - DNA, 43 bp, Chromobacterium violaceum
  misc_feature (20)..(21): n is a, c, g, or t
  misc_feature (22)..(22): k is g, or t
ccgtaacaacctgattatgnnkgcctgcggcgatcacatcgtg

SEQ ID NO: 11 - DNA, 43 bp, Chromobacterium violaceum
  misc_feature (22)..(22): m is a,or c
  misc_feature (23)..(24): n is a, c, g, or t
cacgatgtgatcgccgcaggcmnncataatcaggttgttacgg

SEQ ID NO: 12 - DNA, 45 bp, Chromobacterium violaceum
  misc_feature (21)..(22): n is a, c, g, or t
  misc_feature (23)..(23): k is g, or t
gtaacaacctgattatgcgtnnktgcggcgatcacatcgtgtctg

SEQ ID NO: 13 - DNA, 45 bp, Chromobacterium violaceum
  misc_feature (23)..(23): m is a, or c
  misc_feature (24)..(25): n is a, c, g, or t
cagacacgatgtgatcgccgcamnnacgcataatcaggttgttac

SEQ ID NO: 14 - DNA, 42 bp, Chromobacterium violaceum
  misc_feature (20)..(21): n is a, c, g, or t
  misc_feature (22)..(22): k is g, or t
caacctgattatgcgtgccnnkggcgatcacatcgtgtctgc

SEQ ID NO: 15 - DNA, 42 bp, Chromobacterium violaceum
  misc_feature (21)..(21): m is a,or c
  misc_feature (22)..(23): n is a, c, g, or t
gcagacacgatgtgatcgccmnnggcacgcataatcaggttg

SEQ ID NO: 16 - DNA, 43 bp, Chromobacterium violaceum
  misc_feature (21)..(21): m is a, or c
  misc_feature (22)..(23): n is a, c, g, or t
ccgtaaccaacgttaacacamnncaggccagccataccgtcaa

SEQ ID NO: 17 - DNA, 43 bp, Chromobacterium violaceum
  misc_feature (21)..(22): n is a, c, g, or t
  misc_feature (21)..(21): n is a, c, g, t or u
  misc_feature (22)..(22): n is a, c, g, t or u
  misc_feature (23)..(23): k is g, or t
ttgacggtatggctggcctgnnktgtgttaacgttggttacgg

SEQ ID NO: 18 - DNA, 44 bp, Chromobacterium violaceum
  misc_feature (21)..(21): m is a,or c
  misc_feature (22)..(23): n is a, c, g, or t
cagactgggtgaccagaatamnnaaaaccgtggttgaagtcacc

SEQ ID NO: 19 - DNA, 44 bp, Chromobacterium violaceum
  misc_feature (22)..(23): n is a, c, g, or t
  misc_feature (24)..(24): k is g, or t
ggtgacttcaaccacggttttnnktattctggtcacccagtctg

SEQ ID NO: 20 - DNA, 35 bp, Chromobacterium violaceum
  misc_feature (17)..(17): m is a,or c
  misc_feature (18)..(19): n is a, c, g, or t
  misc_feature (18)..(18): n is a, c, g, t or u
  misc_feature (19)..(19): n is a, c, g, t or u
ccagcgtgaacgcctgmnncataccaacaccgcgc

SEQ ID NO: 21 - DNA, 35 bp, Chromobacterium violaceum
  misc_feature (17)..(18): n is a, c, g, or t
  misc_feature (19)..(19): k is g, or t
gcgcggtgttggtatgnnkcaggcgttcacgctgg